European Patent Specification EP 4 103 730 B1, published November 22, 2023. Title: Enzymatic method for preparation of CMP-Neu5Ac. Applicant: Max-Planck-Gesellschaft zur Foerderung der Wissenschaften e.V. The sequence listing filed with the application follows.

SEQUENCE LISTING (9 sequences)

SEQ ID NO: 1 - protein, 392 aa, Trichormus variabilis
  PEPTIDE (1)..(392): AGE family epimerase/isomerase
MGKNLQALAQLYKNALLNDVLPFWENYSLDSEGGYFTCLDRQGKVYDTDKFIWLQNRQVWTFSMLCNQLEKRENWLKIARNGAKFLAQHGRDDEGNWYFALTRGGEPLVQPYNIFSDCFAAMAFSQYALASGEEWSKDVAMQAYNNVLRRKDNPKGKYTKTYPGTRPMKALAVPMILANLTLEMEWLLPQETLENVLAATVQEVMGDFLDQERGLMYENVAPDGSHIDCFEGRLINPGHGIEAMWFIMDIARRKNDSKTINQAVDVVLNILNFAWDNEYGGLYYFMDAAGHPPQQLEWDQKLWWVHLESLVALAMGYRLTGREVCWEWYQKMHDYSWQHFADPEYGEWFGYLNRRGEVLLNLKGGKWKGCFHVPRALYLCWQQFEALSLQSA

SEQ ID NO: 2 - protein, 293 aa, Pasteurella multocida
  PEPTIDE (1)..(293): N-acetylneuraminate lyase (NAL)
MKNLKGIFSALLVSFNADGSINEKGLRQIVRYNIDKMKVDGLYVGGSTGENFMLSTEEKKEIFRIAKDEAKDEIALIAQVGSVNLQEAIELGKYATELGYDSLSAVTPFYYKFSFPEIKHYYDSIIEATGNYMIVYSIPFLTGVNIGVEQFGELYKNPKVLGVKFTAGDFYLLERLKKAYPNHLIWAGFDEMMLPAASLGVDGAIGSTFNVNGVRARQIFELTQAGKLKEALEIQHVTNDLIEGILANGLYLTIKELLKLDGVEAGYCREPMTKELSPEKVAFAKELKAKYLS

SEQ ID NO: 3 - protein, 228 aa, Neisseria meningitidis (group B)
  PEPTIDE (1)..(228): N-acylneuraminate cytidylyltransferase (CSS)
MEKQNIAVILARQNSKGLPLKNLRKMNGISLLGHTINAAISSKCFDRIIVSTDGGLIAEEAKNFGVEVVLRPAELASDTASSISGVIHALETIGSNSGTVTLLQPTSPLRTGAHIREAFSLFDEKIKGSVVSACPMEHHPLKTLLQINNGEYAPMRHLSDLEQPRQQLPQAFRPNGAIYINDTASLIANNCFFIAPTKLYIMSHQDSIDIDTELDLQQAENILNHKES

SEQ ID NO: 4 - protein, 213 aa, Escherichia coli
  PEPTIDE (1)..(213): Uridine kinase (UDK)
MTDQSHQCVIIGIAGASASGKSLIASTLYRELREQVGDEHIGVIPEDCYYKDQSHLSMEERVKTNYDHPSAMDHSLLLEHLQALKRGSAIDLPVYSYVEHTRMKETVTVEPKKVIILEGILLLTDARLRDELNFSIFVDTPLDICLMRRIKRDVNERGRSMDSVMAQYQKTVRPMFLQFIEPSKQYADIIVPRGGKNRIAIDILKAKISQFFE

SEQ ID NO: 5 - protein, 202 aa, Arabidopsis thaliana [sequence omitted]

SEQ ID NO: 6 - protein, 301 aa, Ruegeria pomeroyi
  PEPTIDE (1)..(301): Polyphosphate:NDP phosphotransferase 3 (PPK3)
MNRNGSTKDPRRMTGAATGEISRYFNDKAPKDIRRAIEKADKDDILSTTYPYDAEMTAKDYRAQMEALQIELVKLQAWIKQSGARVALLFEGRDAAGKGGTIKRFRENLNPRGARVVALSKPTEAERSQWYFQRYIQHLPSAGELVFYDRSWYNRGVVEHVFGWCDEEQRERFFRQVMPFEHDLVDDGIHLFKFWLNVGRAEQLRRFHDRERDPLKQWKLSPVDIAGLDKWEAYTTAISQTLTRSHSDRAPWTVIRSDDKKRARLAAIRTVLSGIDYDNKDRAAVGQPDAAICGGPDIWDA

SEQ ID NO: 7 - protein, 175 aa, Pasteurella multocida
  PEPTIDE (1)..(175): Inorganic pyrophosphatase (PPA)
MGLETVPAGKALPDDIYVVIEIPANSDPIKYEVDKESGALFVDRFMATAMFYPANYGYVNNTLSLDGDPVDVLVPTPYPLQPGSVIRCRPVGVLKMTDEAGSDAKVVAVPHSKLTKEYDHIKDVNDLPALLKAQIQHFFESYKALEAGKWVKVDGWEGVDAARQEILDSFERAKK

SEQ ID NO: 8 - protein, 505 aa, Pseudomonas aeruginosa
  PEPTIDE (1)..(505): Polyphosphate: AMP phosphotransferase (2D-PPK2)
MVFESAEVGHSIDKDTYEKAVIELREALLEAQFELKQQARFPVIILINGIEGAGKGETVKLLNEWMDPRLIEVQSFLRPSDEELERPPQWRFWRRLPPKGRTGIFFGNWYSQMLYARVEGHIKEAKLDQAIDAAERFERMLCDEGALLFKFWFHLSKKQLKERLKALEKDPQHSWKLSPLDWKQSEVYDRFVHYGERVLRRTSRDYAPWYVVEGADERYRALTVGRILLEGLQAALATKERAKRQPHAAPLVSSLDNRGLLDSLDLGQYLDKDAYKEQLAAEQARLAGLIRDKRFRQHSLVAVFEGNDAAGKGGAIRRVTDALDPRQYHIVPIAAPTEEERAQPYLWRFWRHIPARRQFTIFDRSWYGRVLVERIEGFCAPADWLRAYGEINDFEEQLSEYGIIVVKFWLAIDKQTQMERFKEREKTPYKRYKITEEDWRNRDKWDQYVDAVGDMVDRTSTEIAPWTLVEANDKRFARVKVLRTINDAIEAAYKKDKLEHHHHHH

SEQ ID NO: 9 - protein, 324 aa, Pseudomonas aeruginosa
  PEPTIDE (1)..(324): Polyphosphate:ADP phosphotransferase (1D-PPK2)
MGSSHHHHHHSSGLVPRGSHMDSYGDTSGRIGRDWLDRHDEELEQELLDDELNLDELFGPEQEDAPGELSRRRYFRELFRLQRELVKLQNWVVHTGHKVVILFEGRDAAGKGGVIKRITQRLNPRVCRVAALPAPNDREQTQWYFQRYVSHLPAGGEIVLFDRSWYNRAGVERVMGFCNDEQYEEFFRSVPEFEKMLARSGIQLLKYWFSISDAEQHLRFLSRIHDPLKQWKLSPMDLESRRRWEAYTKAKETMLERTHIPEAPWWVVQADDKKRARLNCIHHLLQQMPYREVPQPPVHLPERLRHADYVRHPTPGEIIVPEVY